European Patent Specification EP 3 201 341 B1, published June 25, 2025. Title: HYPERSENSITIVE RESPONSE ELICITOR PEPTIDES AND USE THEREOF. Applicant: Plant Health Care, Inc. The sequence listing filed with the application follows.

SEQUENCE LISTING (232 sequences)

SEQ ID NO: 1 - protein, 23 aa, Artificial
  P1/P4 consensus
  MISC_FEATURE (1)..(1): X at position 1 is optional, S, N, D, isoD, G, A, or S
  MISC_FEATURE (2)..(2): X at position 2 is optional, Q, E, g-glutamate, G, A, or S
  MISC_FEATURE (8)..(8): X at position 8 is Q, E, g-glutamate, G, A, or S
  MISC_FEATURE (9)..(9): X at position 9 is L, I, F, or V
  MISC_FEATURE (10)..(10): X at position 10 is optional, D or isoD
  MISC_FEATURE (11)..(11): X at position 11 is Q, E, g-glutamate, G, A, or S
  MISC_FEATURE (12)..(12): X at position 12 is M, L, I, or F
  MISC_FEATURE (13)..(13): X at position 13 is M, L, I
  MISC_FEATURE (14)..(14): X at position 14 is optional, any hydrophilic amino acid, preferably C, S, T, A, D, isoD, K, or Q
  MISC_FEATURE (15)..(15): X at position 15 is Q, E, g-glutamate, G, A, S, K, or I
  MISC_FEATURE (16)..(16): X at position 16 is M, L, I, V, F
  MISC_FEATURE (17)..(17): X at position 17 is M, L, I, A, or V
  MISC_FEATURE (18)..(18): X at position 18 is Q, E, g-glutamate, G, A, S, M, T, or K
  MISC_FEATURE (19)..(19): X at position 19 is A, D, isoD, S, V, T, K, R, E, H, or G
  MISC_FEATURE (20)..(20): X at position 20 is M, L, or I
  MISC_FEATURE (21)..(21): X at position 21 is M, L, I, V, S, or F
  MISC_FEATURE (22)..(22): X at position 22 is Q, E, g-glutamate, G, A, or S
  MISC_FEATURE (23)..(23): X at position 23 is P, Q, E, g-glutamate, G, A, or S
XXGISEKXXXXXXXXXXXXXXXX

SEQ ID NO: 2 - protein, 23 aa, Artificial
  P4 consensus
  MISC_FEATURE (2)..(2): X at position 2 is Q, E, g-glutamate, G, A, or S
  MISC_FEATURE (8)..(8): X at position 8 is Q, E, g-glutamate, G, A, or S
  MISC_FEATURE (9)..(9): X at position 9 is L, A, D, isoD, I, F, or V
  MISC_FEATURE (11)..(11): X at position 11 is Q, E, g-glutamate, G, A, or S
  MISC_FEATURE (12)..(12): X at position 12 is L, D, isoD, I, or F
  MISC_FEATURE (13)..(13): X at position 13 is L, I, V, or F
  MISC_FEATURE (14)..(14): X at position 14 is any hydrophilic amino acid, preferably C, S, or T
  MISC_FEATURE (15)..(15): X at position 15 is Q, E, g-glutamate, G, A, S, K, or I
  MISC_FEATURE (16)..(16): X at position 16 is L, A, I, V, M, or F
  MISC_FEATURE (17)..(17): X at position 17 is I, S, or F
  MISC_FEATURE (18)..(18): X at position 18 is Q, E, g-glutamate, G, A, S
  MISC_FEATURE (20)..(20): X at position 20 is L, I, V, F
  MISC_FEATURE (21)..(21): X at position 21 is L or F
  MISC_FEATURE (22)..(22): X at position 22 is Q, E, g-glutamate, G, A, or S
SXGISEKXXDXXXXXXXXAXXXP

SEQ ID NO: 3 - protein, 23 aa, Artificial
  P1 consensus
  MISC_FEATURE (1)..(1): X at position 1 is N, D, isoD, G, A, or S
  MISC_FEATURE (2)..(2): X at position 2 is Q, E, g-glutamate, G, A, or S
  MISC_FEATURE (8)..(8): X at position 8 is Q, E, g-glutamate, G, A, or S
  MISC_FEATURE (11)..(11): X at position 11 is Q, E, g-glutamate, G, A, or S
  MISC_FEATURE (15)..(15): X at position 15 is Q, E, g-glutamate, G, A, S
  MISC_FEATURE (18)..(18): X at position 18 is M, T, K, E, g-glutamate, G, A, or S
  MISC_FEATURE (22)..(22): X at position 22 is Q, E, g-glutamate, G, A, or S
  MISC_FEATURE (23)..(23): X at position 23 is Q, E, g-glutamate, G, A, or S
XXGISEKXLDXLLTXLIXALLXX

SEQ ID NO: 4 - protein, 23 aa, Artificial
  P1
NQGISEKQLDQLLTQLIMALLQQ

SEQ ID NO: 5 - protein, 23 aa, Artificial
  P4
SQGISEKQLDQLLCQLIQALLQP

SEQ ID NO: 6 - protein, 23 aa, Artificial
  P4-14S
SQGISEKQLDQLLSQLIQALLQP

SEQ ID NO: 7 - protein, 23 aa, Artificial
  P4-14S-18S
SQGISEKQLDQLLSQLISALLQP

SEQ ID NO: 8 - protein, 23 aa, Artificial
  P4-14S-2,18E
SEGISEKQLDQLLSQLIEALLQP

SEQ ID NO: 9 - protein, 23 aa, Artificial
  P4-2E-8E
SEGISEKELDQLLSQLIQALLQP

SEQ ID NO: 10 - protein, 23 aa, Artificial
  P4-2E-8E-15E
SEGISEKELDQLLSELIQALLQP

SEQ ID NO: 11 - protein, 23 aa, Artificial
  P4-allE
SEGISEKELDELLSELIEALLQP

SEQ ID NO: 12 - protein, 14 aa, Artificial
  P15/20 min consensus
  MISC_FEATURE (7)..(7): X of position 7 is optional, any amino acid
  MISC_FEATURE (10)..(10): X at position 10 is M, E, g-glutamate, G, A, S, T, or K
  MISC_FEATURE (14)..(14): X at position 14 is optional, Q, E, g-glutamate, G, A, S
IAKLISXLIXSLLX

SEQ ID NO: 13 - protein, 19 aa, Artificial
  P14d consensus
  MISC_FEATURE (1)..(1): X at position 1 is Q,N, D, E, g-glutamate, isoD, or S
  MISC_FEATURE (2)..(2): X at position 2 can be D, E, g-glutamate, isoD
  MISC_FEATURE (3)..(3): X at position 3 can be P, D, E, isoD, or g-glutamate
  MISC_FEATURE (4)..(4): X at position 4 can be M, A, S, D, E, isoD, or g-glutamate
  MISC_FEATURE (5)..(5): X at position 5 can be Q, E, or g-glutamate
  MISC_FEATURE (6)..(6): X at position 6 can be A, E, or g-glutamate
  MISC_FEATURE (8)..(8): X at position 8 can be M, L, E, Q, D, N, G, A, S, isoD, or g-glutamate
  MISC_FEATURE (9)..(9): X at position 9 can be Q, N, E, D, G, A, S, isoD or, g-glutamate
  MISC_FEATURE (12)..(12): X at position 12 can be Q, N, E, D, G, A, S, isoD or, g-glutamate
  MISC_FEATURE (13)..(13): X at position 13 can be Q, N, E, D, G, A, S, isoD or, g-glutamate
  MISC_FEATURE (16)..(16): X at position 16 can be K, Q, N, E, D, R, G, A, or S
XXXXXXLXXLLXXLVXLLK

SEQ ID NO: 14 - protein, 13 aa, Artificial
  P14d min consensus
  MISC_FEATURE (2)..(2): X at position 2 can be M, L, E, Q, D, N, G, A, S, isoD, or g-glutamate
  MISC_FEATURE (3)..(3): X at position 3 can be Q, N, E, D, G, A, S, isoD or, g-glutamate
  MISC_FEATURE (6)..(6): X at position 6 is Q, N, E, D, G, A, S, isoD or, g-glutamate
  MISC_FEATURE (7)..(7): X at position 7 can be Q, N, E, D, G, A, S, isoD or, g-glutamate
  MISC_FEATURE (10)..(10): X at position 10 can be K, Q, N, E, D, R, G, A, or S
LXXLLXXLVXLLK

SEQ ID NO: 15 - protein, 14 aa, Artificial
  P3min consensus
  MISC_FEATURE (1)..(1): X at position 1 is L or M
  MISC_FEATURE (2)..(2): X at position 2 can be Q, N, E, g-glutamate, D, isoD, T, S, A, or G
  MISC_FEATURE (3)..(3): X at position 3 can be Q, N, E, g-glutamate, D, isoD, T, S, A, or G
  MISC_FEATURE (6)..(6): X at position 6 can be K, Q, N, E, g-glutamate, D, isoD, T, S, A, or G
  MISC_FEATURE (7)..(7): X at position 7 is L or M
  MISC_FEATURE (9)..(9): X at position 9 can be E, g-glutamate, D, isoD, Q, N, T, S, A, or G
  MISC_FEATURE (10)..(10): X at position 10 can be A, G, S, T, E, g-glutamate, D, isoD, Q, or N
  MISC_FEATURE (12)..(12): X at position 12 is L or M
  MISC_FEATURE (13)..(13): X at position 13 can be Q, N, E, g-glutamate, D, isoD, T, S, A, or G
  MISC_FEATURE (14)..(14): X at position 14 can be Q, N, E, g-glutamate, D, isoD, T, S, A, or G
XXXLLXXFXXIXXX

SEQ ID NO: 16 - protein, 12 aa, Artificial
  P25 consensus
  MISC_FEATURE (2)..(2): X at position 2 can be Q, N, E, g-glutamate, D, isoD, T, S, A, or G
  MISC_FEATURE (3)..(3): X at position 3 can be K, Q, N, E, g-glutamate, D, isoD, T, S, A, or G
  MISC_FEATURE (5)..(5): X at position 5 can be L or M
  MISC_FEATURE (6)..(6): X at position 6 can be K, Q, N, E, g-glutamate, D, isoD, T, S, A, or G
  MISC_FEATURE (9)..(9): X at position 9 can be E, g-glutamate, D, isoD, Q, N, T, S, A, or G
  MISC_FEATURE (10)..(10): X at position 10 can be A, G, S, T, E, g-glutamate, D, isoD, Q, or N
LXXLXXILXXLV

SEQ ID NO: 17 - protein, 16 aa, Artificial
  P25 consensus
  MISC_FEATURE (2)..(2): X at position 2 can be T, S, A, G, D, isoD, E, g-glutamate, Q, or N
  MISC_FEATURE (3)..(3): X at position 3 can be G, T, S, A, D, isoD, E, g-glutamate, Q, or N
  MISC_FEATURE (6)..(6): X at position 6 can be Q, N, E, g-glutamate, D, isoD, T, S, A, or G
  MISC_FEATURE (7)..(7): X at position 7 can be K, Q, N, E, g-glutamate, D, isoD, T, S, A, or G
  MISC_FEATURE (9)..(9): X at position 9 can be L or M
  MISC_FEATURE (10)..(10): X at position 10 can be K, Q, N, E, g-glutamate, D, isoD, T, S, A, or G
  MISC_FEATURE (13)..(13): X at position 13 can be E, g-glutamate, D, isoD, Q, N, T, S, A, or G
  MISC_FEATURE (14)..(14): X at position 14 can be A, G, S, T, E, g-glutamate, D, isoD, Q, or N
  MISC_FEATURE (16)..(16): V at position 16 is optional
LXXVLXXLXXILXXLV

SEQ ID NO: 18 - protein, 27 aa, Artificial
  P17/18
  MISC_FEATURE (1)..(1): X at position 1 can be any amino acid, but preferably Q, S, E, g-glutamate, A, T, G, D, isoD, N, K, or R
  MISC_FEATURE (2)..(2): X at position 2 can be any amino acid, but preferably Q, S, E, g-glutamate, A, T, G, D, isoD, N, K, or R
  MISC_FEATURE (3)..(3): X at position 3 can be any amino acid, but preferably P, Q, S, E, g-glutamate, A, T, G, D, isoD, N, K, or R
  MISC_FEATURE (4)..(4): X at position 4 can be any amino acid, but preferably I, Q, S, E, g-glutamate, A, T, G, D, N, isoD, K, or R
  MISC_FEATURE (5)..(5): X at position 5 can be any amino acid, but preferably D, isoD, S, E, g-glutamate, A, T, G, N, Q, K, or R
  MISC_FEATURE (6)..(6): X at position 6 can be any amino acid, but preferably R, Q, S, E, g-glutamate, A, T, G, D, isoD, N, or K
  MISC_FEATURE (7)..(7): X of position 7 can be any amino acid, but preferably Q, S, E, g-glutamate, A, T, G, D, isoD, N, K, or R
  MISC_FEATURE (8)..(8): X at position 8 can be any amino acid, but preferably T, Q, S, E, g-glutamate, A, G, D, isoD, N, K, or R
  MISC_FEATURE (9)..(9): X at position 9 can be any amino acid, but preferably I, Q, S, E, g-glutamate,  A, T, G, D, isoD, N, K, or R
  MISC_FEATURE (10)..(10): X at position 10 can be any amino acid, but preferably E, g-glutamate, Q, S, A, T, G, D, isoD, N, K, or R
  MISC_FEATURE (11)..(11): X at position 11 can be any amino acid, but preferably Q, S, E, g-glutamate, A, T, G, D, isoD, N, K, or R
  MISC_FEATURE (12)..(12): X at position 12 can be L or M
  MISC_FEATURE (13)..(13): X at position 13 can be any amino acid, but preferably A, S, T, G, D, isoD, E, g-glutamate, Q, N, K, or R
  MISC_FEATURE (14)..(14): X at position 14 can be any amino acid, but preferably Q, A, S, T, G, D, isoD, E, g-glutamate, N, K, or R
  MISC_FEATURE (17)..(17): X at position 17 can be any amino acid, but preferably A, S, T, G, D, isoD, E, g-glutamate, Q, N, K, or R
  MISC_FEATURE (18)..(18): X at position 18 can be any amino acid, but preferably Q, A, S, T, G, D, isoD, E, g-glutamate, N, K, or R
  MISC_FEATURE (21)..(21): X at position 21 can be any amino acid, but preferably K, A, S, T, G, D, isoD, E, g-glutamate, Q, N, or R
  MISC_FEATURE (22)..(22): X at position 22 can be any amino acid, but preferably S, A,T, G, D, isoD, E, g-glutamate, Q, N, K, or R
  MISC_FEATURE (25)..(25): X at position 25 can be any amino acid, but preferably S, A, T, G, D, isoD, E, g-glutamate, Q, N, K, or R
  MISC_FEATURE (26)..(26): X at position 26 can be any amino acid, but preferably P, S, A, T, G, D, isoD, E, g-glutamate, Q, N, K, or R
  MISC_FEATURE (27)..(27): X at position 27 can be any amino acid, but preferably Q, S, A, T, G, D, isoD, E, g-glutamate, N, K, or R
XXXXXXXXXXXXXXLLXXLLXXLLXXX

SEQ ID NO: 19 - protein, 23 aa, Artificial
  P4-14s-9v
SQGISEKQVDQLLSQLIQALLQP

SEQ ID NO: 20 - protein, 23 aa, Artificial
  P4-14s-9F
SQGISEKQFDQLLSQLIQALLQP

SEQ ID NO: 21 - protein, 27 aa, Artificial
  P17/18
  MISC_FEATURE (1)..(1): X at position 1 can be any amino acid, but preferably Q, S, E, g-glutamate, A, T, G, D, isoD, N, K, or R
  MISC_FEATURE (2)..(2): X at position 2 can be any amino acid, but preferably Q, S, E, g-glutamate, A, T, G, D, isoD, N, K, or R
  MISC_FEATURE (3)..(3): X at position 3 can be any amino acid, but preferably P, Q, S, E, g-glutamate, A, T, G, D, isoD, N, K, or R
  MISC_FEATURE (4)..(4): X at position 4 can be any amino acid, but preferably I, Q, S, E, g-glutamate, A, T, G, D, N, isoD, K, or R
  MISC_FEATURE (5)..(5): X at position 5 can be any amino acid, but preferably D, isoD, S, E, g-glutamate, A, T, G, N, Q, K, or R
  MISC_FEATURE (6)..(6): X at position 6 can be any amino acid, but preferably R, Q, S, E, g-glutamate, A, T, G, D, isoD, N, or K
  MISC_FEATURE (7)..(7): X of position 7 can be any amino acid, but preferably Q, S, E, g-glutamate, A, T, G, D, isoD, N, K, or R
  MISC_FEATURE (8)..(8): X at position 8 can be any amino acid, but preferably T, Q, S, E, g-glutamate, A, G, D, isoD, N, K, or R
  MISC_FEATURE (9)..(9): X at position 9 can be any amino acid, but preferably I, Q, S, E, g-glutamate,  A, T, G, D, isoD, N, K, or R
  MISC_FEATURE (10)..(10): X at position 10 can be any amino acid, but preferably E, g-glutamate, Q, S, A, T, G, D, isoD, N, K, or R
  MISC_FEATURE (11)..(11): X at position 11 can be any amino acid, but preferably Q, S, E, g-glutamate, A, T, G, D, isoD, N, K, or R
  MISC_FEATURE (12)..(12): X at position 12 can be L or M
  MISC_FEATURE (13)..(13): X at position 13 can be any amino acid, but preferably A, S, T, G, D, isoD, E, g-glutamate, Q, N, K, or R
  MISC_FEATURE (14)..(14): X at position 14 can be any amino acid, but preferably Q, A, S, T, G, D, isoD, E, g-glutamate, N, K, or R
  MISC_FEATURE (17)..(17): X at position 17 can be any amino acid, but preferably A, S, T, G, D, isoD, E, g-glutamate, Q, N, K, or R
  MISC_FEATURE (18)..(18): X at position 18 can be any amino acid, but preferably Q, A, S, T, G, D, isoD, E, g-glutamate, N, K, or R
  MISC_FEATURE (21)..(21): X at position 21 can be any amino acid, but preferably K, A, S, T, G, D, isoD, E, g-glutamate, Q, N, or R
  MISC_FEATURE (22)..(22): X at position 22 can be any amino acid, but preferably S, A,T, G, D, isoD, E, g-glutamate, Q, N, K, or R
  MISC_FEATURE (25)..(25): X at position 25 can be any amino acid, but preferably S, A, T, G, D, isoD, E, g-glutamate, Q, N, K, or R
  MISC_FEATURE (26)..(26): X at position 26 can be any amino acid, but preferably P, S, A, T, G, D, isoD, E, g-glutamate, Q, N, K, or R
  MISC_FEATURE (27)..(27): X at position 27 can be any amino acid, but preferably Q, S, A, T, G, D, isoD, E, g-glutamate, N, K, or R
XXXXXXXXXXXXXXLLXXLLXXLLXXX

SEQ ID NO: 22 - protein, 23 aa, Artificial
  P4-14s-12i
SQGISEKQLDQILSQLIQALLQP

SEQ ID NO: 23 - protein, 23 aa, Artificial
  P4-14s-12f
SQGISEKQLDQFLSQLIQALLQP

SEQ ID NO: 24 - protein, 23 aa, Artificial
  P4-14s-13i
SQGISEKQLDQLISQLIQALLQP

SEQ ID NO: 25 - protein, 13 aa, Artificial
  P17/18 min consensus
  MISC_FEATURE (1)..(1): X at position 1 can be L or M
  MISC_FEATURE (2)..(2): X at position 2 can be any amino acid, but preferably A, S, T, G, D, isoD, E, g-glutamate, Q, N, K, or R
  MISC_FEATURE (3)..(3): X at position 3 can be any amino acid, but preferably Q, A, S, T, G, D, isoD, E, g-glutamate, N, K, or R
  MISC_FEATURE (6)..(6): X at position 6 can be any amino acid, but preferably A, S, T, G, D, isoD, E, g-glutamate, Q, N, K, or R
  MISC_FEATURE (7)..(7): X at position 7 can be any amino acid, but preferably Q, A, S, T, G, D, isoD, E, g-glutamate, N, K, or R
  MISC_FEATURE (10)..(10): X at position 10 can be any amino acid, but preferably K, A, S, T, G, D, isoD, E, g-glutamate, Q, N, or R
  MISC_FEATURE (11)..(11): X at position 11 can be any amino acid, but preferably S, A,T, G, D, isoD, E, g-glutamate, Q, N, K, or R
XXXLLXXLLXXLL

SEQ ID NO: 26 - protein, 13 aa, Artificial
  P19 consensus
  MISC_FEATURE (1)..(1): X at position 1 is optional and can be L, I, V, F, or M
  MISC_FEATURE (3)..(3): X at position 3 can be any amino acid, but preferably K, A, S, T, G, D, isoD, E, g-glutamate, Q, N, or R
  MISC_FEATURE (4)..(4): X at position 4 can be any amino acid, but preferably A, S, T, G, D, isoD, E, g-glutamate, Q, N, K, or R
  MISC_FEATURE (5)..(5): X at position 5 can be L or M
  MISC_FEATURE (7)..(7): X at position 7 can be any amino acid, but preferably K, A, S, T, G, D, isoD, E, g-glutamate, Q, N, or R
  MISC_FEATURE (10)..(10): X at position 10 can be any amino acid, but preferably A, S, T, G, D, isoD, E, g-glutamate, Q, N, K, or R
  MISC_FEATURE (11)..(11): X at position 11 can be any amino acid, but preferably R, A, S, T, G, D, isoD, E, g-glutamate, Q, N, or K
  MISC_FEATURE (12)..(12): X at position 12 can be L, I, V, F, or M
  MISC_FEATURE (13)..(13): X at position 13 can be L, I, V, F, or M
XLXXXLXLIXXXX

SEQ ID NO: 27 - protein, 23 aa, Artificial
  P4-14s-15a
SQGISEKQLDQLLSALIQALLQP

SEQ ID NO: 28 - protein, 23 aa, Artificial
  P4-14s-15k
SQGISEKQLDQLLSKLIQALLQP

SEQ ID NO: 29 - protein, 23 aa, Artificial
  P4-14s-15s
SQGISEKQLDQLLSSLIQALLQP

SEQ ID NO: 30 - protein, 23 aa, Artificial
  P4-14s-15i
SQGISEKQLDQLLSILIQALLQP

SEQ ID NO: 31 - protein, 20 aa, Artificial
  polyE-min2p4
SEEEEELDQLLSQLIQALLQ

SEQ ID NO: 32 - protein, 23 aa, Artificial
  P4-14s-16i
SQGISEKQLDQLLSQIIQALLQP

SEQ ID NO: 33 - protein, 19 aa, Artificial
  polyE-min3P4
SEEEEELDQLLSQLIQALL

SEQ ID NO: 34 - protein, 23 aa, Artificial
  P4-14s-16f
SQGISEKQLDQLLSQFIQALLQP

SEQ ID NO: 35 - protein, 22 aa, Artificial
  P4-NpolyR
RRRRRGGLDQLLSQLIQALLQP

SEQ ID NO: 36 - protein, 22 aa, Artificial
  P4-CpolyR
LDQLLSQLIQALLQPGGRRRRR

SEQ ID NO: 37 - protein, 23 aa, Artificial
  P4-14s-20i
SQGISEKQLDQLLSQLIQAILQP

SEQ ID NO: 38 - protein, 22 aa, Artificial
  P4-NpolyK
KKKKKGGLDQLLSQLIQALLQP

SEQ ID NO: 39 - protein, 22 aa, Artificial
  P4-CpolyK
LDQLLSQLIQALLQPGGKKKKK

SEQ ID NO: 40 - protein, 23 aa, Artificial
  P4-14s-21f
SQGISEKQLDQLLSQLIQALFQP

SEQ ID NO: 41 - protein, 23 aa, Artificial
  P1-2E
NEGISEKQLDQLLTQLIMALLQQ

SEQ ID NO: 42 - protein, 23 aa, Artificial
  P1-18T
NQGISEKQLDQLLTQLITALLQQ

SEQ ID NO: 43 - protein, 23 aa, Artificial
  P1-18E
NQGISEKQLDQLLTQLIEALLQQ

SEQ ID NO: 44 - protein, 23 aa, Artificial
  P1-18A
NQGISEKQLDQLLTQLIAALLQQ

SEQ ID NO: 45 - protein, 23 aa, Artificial
  P1-18K
NQGISEKQLDQLLTQLIKALLQQ

SEQ ID NO: 46 - protein, 23 aa, Artificial
  P1-2E,8E,11E,15E,18E
NEGISEKELDELLTELIEALLQQ

SEQ ID NO: 47 - protein, 22 aa, Artificial
  P15b/P20 consensus
  MISC_FEATURE (3)..(3): X at position 3 is N, D, or isoD
  MISC_FEATURE (6)..(6): X at position 6 is Q, E, g-glutamate, G, A, or S
  MISC_FEATURE (8)..(8): X at position 8 is N, D, or isoD
  MISC_FEATURE (15)..(15): X at position 15 is optional and can be any amino acid
  MISC_FEATURE (18)..(18): X at position 18 is M, E, g-glutamate, G, A, S, T, or K
  MISC_FEATURE (22)..(22): X at position 22 is optional and can be Q, E, g-glutamate, G, A, or S
KPXDSXSXIAKLISXLIXSLLX

SEQ ID NO: 48 - protein, 45 aa, Artificial
  Wildtype P15
QKDVNFGTPDSTVQNPQDASKPNDSQSNIAKLISALIMSLLQMLT

SEQ ID NO: 49 - protein, 22 aa, Artificial
  P15b
KPNDSQSNIAKLISALIMSLLQ

SEQ ID NO: 50 - protein, 22 aa, Artificial
  P15b-8D-18E
KPNDSQSDIAKLISALIESLLQ

SEQ ID NO: 51 - protein, 22 aa, Artificial
  P15b-8D-18A
KPNDSQSDIAKLISALIASLLQ

SEQ ID NO: 52 - protein, 22 aa, Artificial
  P15b-8D-18S
KPNDSQSDIAKLISALISSLLQ

SEQ ID NO: 53 - protein, 22 aa, Artificial
  P15b-8D-18T
KPNDSQSDIAKLISALITSLLQ

SEQ ID NO: 54 - protein, 22 aa, Artificial
  P15b-8D-18K
KPNDSQSDIAKLISALIKSLLQ

SEQ ID NO: 55 - protein, 22 aa, Artificial
  P15b-8D-6,18E
KPNDSESDIAKLISALIESLLQ

SEQ ID NO: 56 - protein, 22 aa, Artificial
  P15b-3,8D
KPDDSQSDIAKLISALIMSLLQ

SEQ ID NO: 57 - protein, 22 aa, Artificial
  P15b-3,8D-6E
KPDDSESDIAKLISALIMSLLQ

SEQ ID NO: 58 - protein, 22 aa, Artificial
  P15b-3,8D-18E
KPDDSQSDIAKLISALIESLLQ

SEQ ID NO: 59 - protein, 22 aa, Artificial
  P15b-3,8D-6,18E
KPDDSESDIAKLISALIESLLQ

SEQ ID NO: 60 - protein, 22 aa, Artificial
  P15b-3,8D-allE
KPDDSESDIAKLISALIESLLE

SEQ ID NO: 61 - protein, 22 aa, Artificial
  P15b-8D-allE
KPNDSESDIAKLISALIESLLE

SEQ ID NO: 62 - protein, 22 aa, Artificial
  P15b-3D-allE
KPDDSESNIAKLISALIESLLE

SEQ ID NO: 63 - protein, 39 aa, Artificial
  P15a
NFGTPDSTVQNPQDASKPNDSQSNIAKLISALIMSLLQM

SEQ ID NO: 64 - protein, 23 aa, Artificial
  P15
KPNDSQSNIAKLISALIMSLLQM

SEQ ID NO: 65 - protein, 34 aa, Artificial
  P20
GTPDSTVQNPQDASKPNDSQSNIAKLISLIMSLL

SEQ ID NO: 66 - protein, 20 aa, Artificial
  P6/6a consensus
  MISC_FEATURE (4)..(4): X at position 4 is F or Y
  MISC_FEATURE (6)..(6): X at position 6 is Q, E, g-glutamate, G, A, or S
  MISC_FEATURE (7)..(7): X at position 7 is optional and can be M, E, g-glutamate, G, A, S, T, or K or L
  MISC_FEATURE (9)..(9): X at position 9 is M, E, g-glutamate, G, A, S, T, or K
  MISC_FEATURE (10)..(10): X at position 10 is H or N
  MISC_FEATURE (14)..(14): X at position 14 is E, g-glutamate, D, or isoD
  MISC_FEATURE (17)..(17): X at position 17 is Q, E, g-glutamate, G, A, or S
  MISC_FEATURE (19)..(19): X at position 19 is Q, E, g-glutamate, G, A, or S
PSPXTXXLXXIVGXILXAXN

SEQ ID NO: 67 - protein, 20 aa, Artificial
  P6a
PSPFTQMLMHIVGEILQAQN

SEQ ID NO: 68 - protein, 19 aa, Artificial
  P6
PSPFTQLMHIVGEILQAQN

SEQ ID NO: 69 - protein, 20 aa, Artificial
  P6a-7A
PSPFTQALMHIVGEILQAQN

SEQ ID NO: 70 - protein, 20 aa, Artificial
  P6a-10N
PSPFTQMLMNIVGEILQAQN

SEQ ID NO: 71 - protein, 20 aa, Artificial
  P6a-4Y
PSPYTQMLMHIVGEILQAQN

SEQ ID NO: 72 - protein, 20 aa, Artificial
  P6a-14D
PSPFTQMLMHIVGDILQAQN

SEQ ID NO: 73 - protein, 20 aa, Artificial
  P6a-7,9A
PSPFTQALAHIVGEILQAQN

SEQ ID NO: 74 - protein, 20 aa, Artificial
  P6a-6E-7A
PSPFTEALMHIVGEILQAQN

SEQ ID NO: 75 - protein, 20 aa, Artificial
  P6a-6,17E-7A
PSPFTEALMHIVGEILEAQN

SEQ ID NO: 76 - protein, 20 aa, Artificial
  P6a-allE-7A
PSPFTEALMHIVGEILEAEN

SEQ ID NO: 77 - protein, 20 aa, Artificial
  P6a-allE-4Y-7A
PSPYTEALMHIVGEILEAEN

SEQ ID NO: 78 - protein, 20 aa, Artificial
  P6a-allE-7A-10N
PSPFTEALMNIVGEILEAEN

SEQ ID NO: 79 - protein, 20 aa, Artificial
  P6a-allE-7A-14D
PSPFTEALMHIVGDILEAEN

SEQ ID NO: 80 - protein, 20 aa, Artificial
  P6a-allE-4Y-7A-10N-14D
PSPYTEALMNIVGDILEAEN

SEQ ID NO: 81 - protein, 50 aa, Artificial
  P17
TSSSPGLFQSGGDNGLGGHNANSALGQQPIDRQTIEQMAQLLAQLLKSLL

SEQ ID NO: 82 - protein, 50 aa, Artificial
  P17a
TSSSPGLFQSGGDNGLGGHNANSALGQQPIDRQTIEQLAQLLAQLLKSLL

SEQ ID NO: 83 - protein, 27 aa, Artificial
  P18
QQPIDRQTIEQMAQLLAQLLKSLLSPQ

SEQ ID NO: 84 - protein, 27 aa, Artificial
  P18a
QQPIDRQTIEQLAQLLAQLLKSLLSPQ

SEQ ID NO: 85 - protein, 16 aa, Artificial
  P18b
IEQMAQLLAQLLKSLL

SEQ ID NO: 86 - protein, 16 aa, Artificial
  P18c
IEQLAQLLAQLLKSLL

SEQ ID NO: 87 - protein, 20 aa, Artificial
  P18d
DRQTIEQMAQLLAQLLKSLL

SEQ ID NO: 88 - protein, 20 aa, Artificial
  P18e
DRQTIEQLAQLLAQLLKSLL

SEQ ID NO: 89 - protein, 25 aa, Artificial
  amino acids 116 to 140 of the full length Erwinia amylovora HrpW (P19)
ITPDGQGGGQIGDNPLLKAMLKLIA

SEQ ID NO: 90 - protein, 25 aa, Artificial
  P19-20L
ITPDGQGGGQIGDNPLLKALLKLIA

SEQ ID NO: 91 - protein, 30 aa, Artificial
  P19a
ITPDGQGGGQIGDNPLLKAMLKLIARMMDG

SEQ ID NO: 92 - protein, 30 aa, Artificial
  P19a-allL
ITPDGQGGGQIGDNPLLKALLKLIARLLDG

SEQ ID NO: 93 - protein, 13 aa, Artificial
  HR Box Peptide Consensus
  MISC_FEATURE (1)..(1): X at position 1 is L, I, V, or F
  MISC_FEATURE (2)..(2): X at position 2 is optional and, when present, is any amino acid
  MISC_FEATURE (3)..(3): X at position 3 is any amino acid
  MISC_FEATURE (4)..(4): X at position 4 is L, I, V, or F
  MISC_FEATURE (5)..(5): X at position 5 is L or I
  MISC_FEATURE (6)..(6): X at position 6 is optional and, when present, is any amino acid
  MISC_FEATURE (7)..(7): X at position 7 is any amino acid
  MISC_FEATURE (8)..(8): X at position 8 is L, I, V, or F
  MISC_FEATURE (9)..(9): X at position 9 is L, I, V, or A
  MISC_FEATURE (10)..(10): X at position 10 is optional and, when present, is any amino acid
  MISC_FEATURE (11)..(11): X at position 11 is any amino acid
  MISC_FEATURE (12)..(12): X at position 12 is L or I
  MISC_FEATURE (13)..(13): X at position 13 is L, I, V, or F
XXXXXXXXXXXXX

SEQ ID NO: 94 - protein, 17 aa, Artificial
  P4-14s-dN6
KQLDQLLSQLIQALLQP

SEQ ID NO: 95 - protein, 18 aa, Artificial
  P4-14s-dN5
EKQLDQLLSQLIQALLQP

SEQ ID NO: 96 - protein, 19 aa, Artificial
  P4-14s-dN4
SEKQLDQLLSQLIQALLQP

SEQ ID NO: 97 - protein, 21 aa, Artificial
  P4-14s-dN2
GISEKQLDQLLSQLIQALLQP

SEQ ID NO: 98 - protein, 23 aa, Artificial
  P4-14s-3E
SQEISEKQLDQLLSQLIQALLQP

SEQ ID NO: 99 - protein, 23 aa, Artificial
  P4-14S-4L
SQGLSEKQLDQLLSQLIQALLQP

SEQ ID NO: 100 - protein, 23 aa, Artificial
  P4-14S-4A
SQGASEKQLDQLLSQLIQALLQP

SEQ ID NO: 101 - protein, 23 aa, Artificial
  P4-14S-4D
SQGDSEKQLDQLLSQLIQALLQP

SEQ ID NO: 102 - protein, 23 aa, Artificial
  P4-14s-5V
SQGIVEKQLDQLLSQLIQALLQP

SEQ ID NO: 103 - protein, 23 aa, Artificial
  P4-14s-6R
SQGISRKQLDQLLSQLIQALLQP

SEQ ID NO: 104 - protein, 23 aa, Artificial
  P4-14s-6V
SQGISVKQLDQLLSQLIQALLQP

SEQ ID NO: 105 - protein, 23 aa, Artificial
  P4-14s-7D
SQGISEDQLDQLLSQLIQALLQP

SEQ ID NO: 106 - protein, 23 aa, Artificial
  P4-14s-7V
SQGISEVQLDQLLSQLIQALLQP

SEQ ID NO: 107 - protein, 23 aa, Artificial
  P4-14S-8V
SQGISEKVLDQLLSQLIQALLQP

SEQ ID NO: 108 - protein, 23 aa, Artificial
  P4-14S-8S
SQGISEKSLDQLLSQLIQALLQP

SEQ ID NO: 109 - protein, 23 aa, Artificial
  P1-1S
SQGISEKQLDQLLTQLIMALLQQ

SEQ ID NO: 110 - protein, 23 aa, Artificial
  P1-14S
NQGISEKQLDQLLSQLIMALLQQ

SEQ ID NO: 111 - protein, 23 aa, Artificial
  P4-14S-10V
SQGISEKQLVQLLSQLIQALLQP

SEQ ID NO: 112 - protein, 23 aa, Artificial
  P4-14S-11V
SQGISEKQLDVLLSQLIQALLQP

SEQ ID NO: 113 - protein, 23 aa, Artificial
  P4-14S-12V
SQGISEKQLDQVLSQLIQALLQP

SEQ ID NO: 114 - protein, 23 aa, Artificial
  P4-14S-12S
SQGISEKQLDQSLSQLIQALLQP

SEQ ID NO: 115 - protein, 23 aa, Artificial
  P1-18Q
NQGISEKQLDQLLTQLIQALLQQ

SEQ ID NO: 116 - protein, 23 aa, Artificial
  P4-14S-14V
SQGISEKQLDQLLVQLIQALLQP

SEQ ID NO: 117 - protein, 23 aa, Artificial
  P4-14S-15V
SQGISEKQLDQLLSVLIQALLQP

SEQ ID NO: 118 - protein, 23 aa, Artificial
  P1-23P
NQGISEKQLDQLLTQLIMALLQP

SEQ ID NO: 119 - protein, 23 aa, Artificial
  P4-14s-17L
SQGISEKQLDQLLSQLLQALLQP

SEQ ID NO: 120 - protein, 23 aa, Artificial
  P4-14s-17A
SQGISEKQLDQLLSQLAQALLQP

SEQ ID NO: 121 - protein, 23 aa, Artificial
  P4-14s-17V
SQGISEKQLDQLLSQLVQALLQP

SEQ ID NO: 122 - protein, 23 aa, Artificial
  P4-14S-18V
SQGISEKQLDQLLSQLIVALLQP

SEQ ID NO: 123 - protein, 23 aa, Artificial
  P4-14S-19V
SQGISEKQLDQLLSQLIQVLLQP

SEQ ID NO: 124 - protein, 23 aa, Artificial
  P4-14S-19D
SQGISEKQLDQLLSQLIQDLLQP

SEQ ID NO: 125 - protein, 23 aa, Artificial
  P4-14S-19S
SQGISEKQLDQLLSQLIQSLLQP

SEQ ID NO: 126 - protein, 21 aa, Artificial
  polyE-minP1
SEEEEELDQLLTQLIEALLQQ

SEQ ID NO: 127 - protein, 23 aa, Artificial
  P4-14S-21S
SQGISEKQLDQLLSQLIQALSQP

SEQ ID NO: 128 - protein, 23 aa, Artificial
  P4-14S-21I
SQGISEKQLDQLLSQLIQALIQP

SEQ ID NO: 129 - protein, 23 aa, Artificial
  P4-14S-21V
SQGISEKQLDQLLSQLIQALVQP

SEQ ID NO: 130 - protein, 23 aa, Artificial
  P4-14S-22V
SQGISEKQLDQLLSQLIQALLVP

SEQ ID NO: 131 - protein, 21 aa, Artificial
  P4-14S-dC2
SQGISEKQLDQLLSQLIQALL

SEQ ID NO: 132 - protein, 22 aa, Artificial
  p4-d10
SQGISEKQLQLLSQLIQALLQP

SEQ ID NO: 133 - protein, 22 aa, Artificial
  p4-d14
SQGISEKQLDQLLQLIQALLQP

SEQ ID NO: 134 - protein, 20 aa, Artificial
  polyE-min2P1
SEEEEELDQLLTQLIEALLQ

SEQ ID NO: 135 - protein, 13 aa, Artificial
  P6/6a min consensus
  MISC_FEATURE (1)..(1): X at position 1 is F or Y
  MISC_FEATURE (3)..(3): X at position 3 is Q, E, g-glutamate, G, A, or S
  MISC_FEATURE (4)..(4): X at position 4 is optional and can be M, E, g-glutamate, G, A, S, T, or K, or L
  MISC_FEATURE (6)..(6): X at position 6 is M, E, g-glutamate, G, A, S, T, or K
  MISC_FEATURE (7)..(7): X at position 7 is H or N
  MISC_FEATURE (11)..(11): X at position 11 is E, g-glutamate, D, or isoD
XTXXLXXIVGXIL

SEQ ID NO: 136 - protein, 23 aa, Artificial
  P4-14A
SQGISEKQLDQLLAQLIQALLQP

SEQ ID NO: 137 - protein, 23 aa, Artificial
  p4-14D
SQGISEKQLDQLLDQLIQALLQP

SEQ ID NO: 138 - protein, 23 aa, Artificial
  P4-14K
SQGISEKQLDQLLKQLIQALLQP

SEQ ID NO: 139 - protein, 23 aa, Artificial
  P4-14Q
SQGISEKQLDQLLQQLIQALLQP

SEQ ID NO: 140 - protein, 24 aa, Artificial
  p4-i9A
SQGISEKQALDQLLSQLIQALLQP

SEQ ID NO: 141 - protein, 19 aa, Artificial
  polyE-min3P1
SEEEEELDQLLTQLIEALL

SEQ ID NO: 142 - protein, 39 aa, Artificial
  P15a-34Q-39P
NFGTPDSTVQNPQDASKPNDSQSNIAKLISALIQSLLQP

SEQ ID NO: 143 - protein, 39 aa, Artificial
  P15a-39P
NFGTPDSTVQNPQDASKPNDSQSNIAKLISALIMSLLQP

SEQ ID NO: 144 - protein, 39 aa, Artificial
  P15a-34Q
NFGTPDSTVQNPQDASKPNDSQSNIAKLISALIQSLLQM

SEQ ID NO: 145 - DNA, 69 bp, Artificial
  P4-14s A. thaliana
tctcaaggaatttctgaaaagcaacttgatcaacttctttctcaacttattcaagctcttcttcaacct

SEQ ID NO: 146 - DNA, 69 bp, Artificial
  P4-14s E. coli
agccagggtattagcgaaaaacagctggatcagctgctgagccagctgattcaggcactgctgcagccg

SEQ ID NO: 147 - DNA, 69 bp, Artificial
  P1-2E,8E,11E,15E,18E A. thaliana
aatgaaggaatttctgaaaaggaacttgatgaacttcttactgaacttattgaagctcttcttcaacaa

SEQ ID NO: 148 - DNA, 69 bp, Artificial
  P1-2E,8E,11E,15E,18 E. coli
aatgaaggtattagcgaaaaagaactggatgaactgctgaccgaactgattgaagcactgctgcagcag

SEQ ID NO: 149 - protein, 22 aa, Artificial
  P15-59G
SEEEEEGGIAKLISALIESLLE

SEQ ID NO: 150 - protein, 20 aa, Artificial
  P15-59
SEEEEEIAKLISALIESLLE

SEQ ID NO: 151 - protein, 20 aa, Artificial
  P20-5
KPNDSQSNIAKLISLIMSLL

SEQ ID NO: 152 - protein, 20 aa, Artificial
  P20-6
KPNDSQSNIAKLISLIESLL

SEQ ID NO: 153 - protein, 21 aa, Artificial
  amino acids 85-103 of full-length harpin of Xanthomonas oryzae pv. Oryzae
PSPFTQMLMHIVGEILQAQNG

SEQ ID NO: 154 - protein, 14 aa, Artificial
  motif 2
  MISC_FEATURE (1)..(1): X at position 1 can be P, A, or V
  MISC_FEATURE (3)..(3): X at position 3 can be P, Q, or A
  MISC_FEATURE (4)..(4): X at position 4 can be F, L, or Y
  MISC_FEATURE (7)..(7): X at position 7 can be M or A
  MISC_FEATURE (10)..(10): X at position 10 can be H, N, or Q
  MISC_FEATURE (13)..(13): X at position 13 can be G or M
  MISC_FEATURE (14)..(14): X at position 14 can be E, D, or Q
XSXXTQXLMXIVXX

SEQ ID NO: 155 - protein, 17 aa, Artificial
  P6b
FTQMLMHIVGEILQAQN

SEQ ID NO: 156 - protein, 16 aa, Artificial
  P6c
PSPFTQMLMHIVGEIL

SEQ ID NO: 157 - protein, 20 aa, Artificial
  P6-7L
PSPFTQLLMHIVGEILQAQN

SEQ ID NO: 158 - protein, 20 aa, Artificial
  P6-9E
PSPFTQMLEHIVGEILQAQN

SEQ ID NO: 159 - protein, 20 aa, Artificial
  P6a-7L,9E
PSPFTQLLEHIVGEILQAQN

SEQ ID NO: 160 - protein, 19 aa, Artificial
  P6d
SEEEEEFTQMLMHIVGEIL

SEQ ID NO: 161 - protein, 19 aa, Artificial
  P6d-7L-9E
SEEEEEFTQLLEHIVGEIL

SEQ ID NO: 162 - protein, 50 aa, Artificial
  amino acids 10 to 59 of the full length Erwinia amylovora HrpW
TSSSPGLFQSGGDNGLGGHNANSALGQQPIDRQTIEQMAQLLAELLKSLL

SEQ ID NO: 163 - protein, 24 aa, Artificial
  18-1
QQPIDRQTIEQMAQLLAQLLKSLL

SEQ ID NO: 164 - protein, 22 aa, Artificial
  P18-4
DRQTIEQLAQLLAQLLKSLLSP

SEQ ID NO: 165 - protein, 20 aa, Artificial
  P18-5
QTIEQLAQLLAQLLKSLLSP

SEQ ID NO: 166 - protein, 22 aa, Artificial
  P18-6
SEEEEEIEQLAQLLAQLLKSLL

SEQ ID NO: 167 - protein, 19 aa, Artificial
  P18-7
SEEEEELAQLLAQLLKSLL

SEQ ID NO: 168 - protein, 26 aa, Artificial
  P19-5
SEEEEEIGDNPLLKALLKLIARLLDG

SEQ ID NO: 169 - protein, 26 aa, Artificial
  P19-5a
SEEEEEIGDDELLKALLKLIARLLDG

SEQ ID NO: 170 - protein, 21 aa, Artificial
  P19-6
SEEEEELLKALLKLIARLLDG

SEQ ID NO: 171 - protein, 24 aa, Artificial
  P19-11
SEEEEEIGDNPLLKALLKLIARLL

SEQ ID NO: 172 - protein, 19 aa, Artificial
  P19-7
SEEEEELLKALLKLIARLL

SEQ ID NO: 173 - protein, 18 aa, Artificial
  P19-8
SEEEEELKALLKLIARLL

SEQ ID NO: 174 - protein, 34 aa, Artificial
  amino acids 92 to 125 of the Ralstonia solanacearum PopA
QAPQSANKTGNVDDANNQDPMQALMQLLEDLVKL

SEQ ID NO: 175 - protein, 19 aa, Artificial
  P14d
QDPMQALMQLLEDLVKLLK

SEQ ID NO: 176 - protein, 19 aa, Artificial
  P14e
QDPAQALLQLLEDLVKLLK

SEQ ID NO: 177 - protein, 19 aa, Artificial
  P14f
QDPAQALEQLLEDLVKLLK

SEQ ID NO: 178 - protein, 20 aa, Artificial
  P14-30
SEEEEEALEQLLEDLVKLLK

SEQ ID NO: 179 - protein, 55 aa, Artificial
  amino acids 206 to 260 of the Ralstonia solanacearum  PopA
NGADGGNGVNGNQANGPQNAGDVNGANGADDGSEDQGGLTGVLQKLMKILNALVQ

SEQ ID NO: 180 - protein, 32 aa, Artificial
  P2
ANGADDGSEDQGGLTLTGVLQKLMKILNALVQ

SEQ ID NO: 181 - protein, 24 aa, Artificial
  P25-4
EDQGGLTLTGVLQKLMKILNALVQ

SEQ ID NO: 182 - protein, 19 aa, Artificial
  P25
GGLTLTGVLQKLMKILNAL

SEQ ID NO: 183 - protein, 22 aa, Artificial
  P25s
EDQGGLTLTGVLQKLMKILNAL

SEQ ID NO: 184 - protein, 22 aa, Artificial
  P25-7
EDQGGLTLTGVLQKLLKILNAL

SEQ ID NO: 185 - protein, 22 aa, Artificial
  P25-8
EDQGGLTLTGVLQELMEILNAL

SEQ ID NO: 186 - protein, 24 aa, Artificial
  P25-20E
EDQGGLTLTGVLQKLLKILEALVQ

SEQ ID NO: 187 - protein, 22 aa, Artificial
  P25-10
SEEEELTLTGVLQKLLKILEAL

SEQ ID NO: 188 - protein, 21 aa, Artificial
  P25-11
SEEEEELTGVLQKLLKILEAL

SEQ ID NO: 189 - protein, 16 aa, Artificial
  P30-2
SEELEELLEELIEELL

SEQ ID NO: 190 - protein, 15 aa, Artificial
  P30-3
LEELLEELIEELLEE

SEQ ID NO: 191 - protein, 23 aa, Artificial
  P4-14s-18e
SEGISEKQLDQLLSQLIEALLQP

SEQ ID NO: 192 - protein, 18 aa, Artificial
  minp4-PolyE
LDQLLSQLIQALLEEEEE

SEQ ID NO: 193 - protein, 18 aa, Artificial
  SEE-minp4-EE
SEELDQLLSQLIQALLEE

SEQ ID NO: 194 - protein, 24 aa, Artificial
  P4-7E-CR
SQGISEEQLDQLLSQLIQALLQPR

SEQ ID NO: 195 - protein, 23 aa, Artificial
  p1-allE-17A
NEGISEKELDELLTELAEALLQQ

SEQ ID NO: 196 - protein, 23 aa, Artificial
  P4-14s-9i
SQGISEKQIDQLLSQLIQALLQP

SEQ ID NO: 197 - protein, 20 aa, Artificial
  p6a-dN3-sol
SEEFTQMLMHIVGEILQAQN

SEQ ID NO: 198 - protein, 20 aa, Artificial
  p6a-dC4-sol
SEEEPSPFTQMLMHIVGEIL

SEQ ID NO: 199 - protein, 37 aa, Artificial
  P14c
QAGPQSANKTGNVDDANNQDPMQALMQLLEDLVKLLK

SEQ ID NO: 200 - protein, 22 aa, Artificial
  P25-15
SEEEEELTLTGVLQKLLKILEA

SEQ ID NO: 201 - protein, 19 aa, Artificial
  P25-16
SEEEEEVLQKLLKILEALV

SEQ ID NO: 202 - protein, 19 aa, Artificial
  P25-17
SEEEEELQKLLKILEALVQ

SEQ ID NO: 203 - protein, 44 aa, Artificial
  amino acids 137 to 180 of Erwinia amylovora HrpN
STSQNDDSTSGTDSTSDSSDPMQQLLKMFSEIMQSLFGDGQDGT

SEQ ID NO: 204 - protein, 41 aa, Artificial
  P3
QNDDSTSGTDSTSDSSDPMQQLLKMFSEIMQSLFGDGQDGT

SEQ ID NO: 205 - protein, 19 aa, Artificial
  P3-3
SDPMQQLLKMFSEIMQSLF

SEQ ID NO: 206 - protein, 20 aa, Artificial
  P3-4
SEEELQQLLKLFSEILQSLF

SEQ ID NO: 207 - protein, 21 aa, Artificial
  P3-6
SEEEEELQQLLKLFSEILQSL

SEQ ID NO: 208 - protein, 20 aa, Artificial
  P3-7
SEEEEELQQLLKLFSEILQS

SEQ ID NO: 209 - protein, 20 aa, Artificial
  P3-11
LQQLLKLFSEILQSLFEEEE

SEQ ID NO: 210 - protein, 13 aa, Artificial
  P30-4
LEELLEELIEELL

SEQ ID NO: 211 - protein, 16 aa, Artificial
  P30-1
RLRRLLRRLIRRLLRP

SEQ ID NO: 212 - protein, 15 aa, Artificial
  P30-5
LDDLLDDLIDDLLDD

SEQ ID NO: 213 - protein, 15 aa, Artificial
  P18-13
LEELLEELLEELLEE

SEQ ID NO: 214 - protein, 15 aa, Artificial
  P14-54
LEQLLEDLVKLLKEE

SEQ ID NO: 215 - protein, 15 aa, Artificial
  P14-55
LEQLLEDLVELLEEE

SEQ ID NO: 216 - protein, 15 aa, Artificial
  P14-56
LEELLEDLVELLEEE

SEQ ID NO: 217 - protein, 15 aa, Artificial
  P14-57
LEELLEELVELLEEE

SEQ ID NO: 218 - protein, 18 aa, Artificial
  P3-12
LEELLELFEEILEELFEE

SEQ ID NO: 219 - protein, 18 aa, Artificial
  P3-13
LEELLKLFEEILEELFEE

SEQ ID NO: 220 - protein, 14 aa, Artificial
  P20-50a
IEELIELIEELLEE

SEQ ID NO: 221 - protein, 15 aa, Artificial
  P15-67
IEELIEELIEELLEE

SEQ ID NO: 222 - protein, 14 aa, Artificial
  P19-54c
LEELLKLIERLLEE

SEQ ID NO: 223 - protein, 14 aa, Artificial
  P19-54b
LEELLELIERLLEE

SEQ ID NO: 224 - protein, 14 aa, Artificial
  P19-54a
LEELLKLIEELLEE

SEQ ID NO: 225 - protein, 14 aa, Artificial
  P19-54
LEELLELIEELLEE

SEQ ID NO: 226 - protein, 25 aa, Artificial
  P19-4
QGGGQIGDNPLLKAMLKLIARMMDG

SEQ ID NO: 227 - protein, 18 aa, Artificial
  P15-dN4
SQSNIAKLISALIMSLLQ

SEQ ID NO: 228 - protein, 26 aa, Artificial
  P18-3
QQPIDRQTIEQLAQLLAQLLKSLLSP

SEQ ID NO: 229 - protein, 24 aa, Artificial
  P18-2
QQPIDRQTIEQLAQLLAQLLKSLL

SEQ ID NO: 230 - protein, 44 aa, Artificial; identical to SEQ ID NO: 203
  amino acids 137 to 180 of Erwinia amylovora HrpN

SEQ ID NO: 231 - protein, 19 aa, Artificial
  P18-10
SEEEEELAELLAELLKSLL

SEQ ID NO: 232 - protein, 21 aa, Artificial
  polyE-minP4
SEEEEELDQLLSQLIQALLQP